European Patent Specification EP 3 265 119 B1, published October 11, 2023. Title: SAFE AND EFFECTIVE BETA-LACTAMASE DOSING FOR MICROBIOME PROTECTION. Applicant: Synthetic Biologics, Inc. SLIMAN, Joseph. The sequence listing filed with the application follows.

SEQUENCE LISTING (2 sequences)

SEQ ID NO: 1 - protein, 264 aa, Artificial Sequence
  Synthetic sequence
TEMKDDFAKLEEQFDAKLGIFALDTGTNRTVAYRPDERFAFASTIKALTVGVLLQQKSIEDLNQRITYTRDDLVNYNPITEKHVDTGMTLKELADASLRYSDNAAQNLILKQIGGPESLKKELRKIGDEVTNPERFEPELNEVNPGETQDTSTARALVTSLRAFALEDKLPSEKRELLIDWMKRNTTGDALIRAGVPDGWEVADKTGAASYGTRNDIAIIWPPKGDPVVLAVLSSRDKKDAKYDNKLIAEATKVVMKALNMNGK

SEQ ID NO: 2 - DNA, 795 bp, Artificial Sequence
  Synthetic sequence
atgactgagatgaaagatgattttgcgaagctggaagaacagtttgacgcaaaattgggcattttcgcgttggacacgggtacgaatcgtacggttgcctaccgtccggacgagcgcttcgccttcgcgagcacgatcaaagccctgaccgtcggcgtgctgctccagcaaaagagcatcgaggacctgaaccagcgcattacctacacccgtgatgatctggtgaactataatccgatcaccgagaaacacgttgataccggtatgaccctgaaagaactggcagatgcaagcctgcgctacagcgataacgcggctcagaatctgattctgaagcaaatcggtggtccggagagcttgaagaaagaactgcgtaaaatcggcgatgaagtcactaatccggagcgttttgagccggagctgaacgaagtgaatccgggtgaaacgcaagacacgagcaccgcgcgtgcgcttgtcacctccctgcgcgctttcgcactggaagataagctgccgtcggagaaacgcgagctgctgatcgactggatgaagcgcaatacgaccggcgacgcgctgattcgtgcgggcgttccggacggttgggaagtggctgacaagaccggtgcggcgagctacggcacccgtaacgatatcgcgatcatttggccacctaaaggtgacccggtcgtgctggccgtactgagcagccgtgacaagaaagacgcaaagtatgataacaagctgattgcagaggcgaccaaagttgttatgaaggcactgaacatgaatggtaag